European Patent Specification EP 3 960 188 B1, published April 2, 2025. Title: GENE THERAPY. Applicant: The University of Manchester. Application PCT/GB2018/050347. The sequence listing filed with the application follows.

SEQUENCE LISTING (8 sequences)

SEQ ID NO: 1 - DNA, 1650 bp, Artificial Sequence
  coIDS DNA sequence
atgcctccacctagaactggaagaggcctgctgtggctgggcctggtgctgtctagtgtgtgtgtggccctgggcagcgagacacaggccaacagcacaaccgacgccctgaacgtgctgctgatcatcgtggacgacctgaggcctagcctgggctgctacggcgataagctcgtgcggagccccaacatcgatcagctggcctctcacagcctgctgttccagaacgcattcgcacagcaggcagtgtgcgcccccagcagagtgtctttcctgaccggcagaaggcccgacaccacccggctgtacgacttcaacagctactggcgggtgcacgccggcaacttcagcaccatcccccagtacttcaaagaaaacggctacgtgaccatgagcgtgggcaaggtgttccaccccggcatcagctccaaccacaccgacgacagcccctacagctggtccttcccaccctaccaccccagcagcgagaagtacgagaacaccaagacctgcagaggccccgacggcgagctgcatgccaatctgctgtgccccgtggacgtgctggatgtgcctgagggaaccctgcccgacaagcagtctaccgagcaggccattcagctgctggaaaagatgaagaccagcgccagccccttcttcctggccgtgggctatcacaagccccacatccctttcagataccccaaagagttccagaagctgtaccccctggaaaacatcaccctggcccccgatcctgaggtgccagatggactgcctcccgtggcctacaacccctggatggacatccggcagcgcgaggatgtgcaggccctgaatatcagcgtgccctacggccccatccccgtggatttccagcggaagatccggcagagctacttcgccagcgtgtcctacctggacacccaagtgggcagactgctgagcgccctggacgatctgcagctggccaactccaccatcattgccttcaccagcgaccacggctgggccctgggagaacatggcgagtgggccaagtacagcaacttcgacgtggccacccacgtgcccctgatcttctacgtgccaggcagaaccgccagcctgcctgaggctggcgagaagctgttcccttacctggaccccttcgacagcgcctcccagctgatggaacctggcagacagagcatggacctggtggaactggtgtccctgttccccacactggccggactggctggactgcaggtgccccctagatgtcccgtgcctagctttcacgtggaactgtgcagagagggcaagaacctgctgaagcacttccggttccgggacctggaagaagatccctacctgcccggcaaccccagagagctgatcgcctacagccagtaccccagacccagcgacatccctcagtggaacagcgacaagcccagcctgaaggacatcaagatcatgggctacagcatccggaccatcgactaccggtacaccgtgtgggtgggattcaaccccgacgagttcctggccaatttctccgacatccacgccggggagctgtacttcgtggacagcgatcccctgcaggaccacaacatgtacaacgacagccagggcggcgacctgttccagctgctgatgccc

SEQ ID NO: 2 - DNA, 1650 bp, Homo sapiens
atgccgccaccccggaccggccgaggccttctctggctgggtctggttctgagctccgtctgcgtcgccctcggatccgaaacgcaggccaactcgaccacagatgctctgaacgttcttctcatcatcgtggatgacctgcgcccctccctgggctgttatggggataagctggtgaggtccccaaatattgaccaactggcatcccacagcctcctcttccagaatgcctttgcgcagcaagcagtgtgcgccccgagccgcgtttctttcctcactggcaggagacctgacaccacccgcctgtacgacttcaactcctactggagggtgcacgctggaaacttctccaccatcccccagtacttcaaggagaatggctatgtgaccatgtcggtgggaaaagtctttcaccctgggatatcttctaaccataccgatgattctccgtatagctggtcttttccaccttatcatccttcctctgagaagtatgaaaacactaagacatgtcgagggccagatggagaactccatgccaacctgctttgccctgtggatgtgctggatgttcccgagggcaccttgcctgacaaacagagcactgagcaagccatacagttgttggaaaagatgaaaacgtcagccagtcctttcttcctggccgttgggtatcataagccacacatccccttcagataccccaaggaatttcagaagttgtatcccttggagaacatcaccctggcccccgatcccgaggtccctgatggcctaccccctgtggcctacaacccctggatggacatcaggcaacgggaagacgtccaagccttaaacatcagtgtgccgtatggtccaattcctgtggactttcagcggaaaatccgccagagctactttgcctctgtgtcatatttggatacacaggtcggccgcctcttgagtgctttggacgatcttcagctggccaacagcaccatcattgcatttacctcggatcatgggtgggctctaggtgaacatggagaatgggccaaatacagcaattttgatgttgctacccatgttcccctgatattctatgttcctggaaggacggcttcacttccggaggcaggcgagaagcttttcccttacctcgacccttttgattccgcctcacagttgatggagccaggcaggcaatccatggaccttgtggaacttgtgtctctttttcccacgctggctggacttgcaggactgcaggttccacctcgctgccccgttccttcatttcacgttgagctgtgcagagaaggcaagaaccttctgaagcattttcgattccgtgacttggaagaggatccgtacctccctggtaatccccgtgaactgattgcctatagccagtatccccggccttcagacatccctcagtggaattctgacaagccgagtttaaaagatataaagatcatgggctattccatacgcaccatagactataggtatactgtgtgggttggcttcaatcctgatgaatttctagctaacttttctgacatccatgcaggggaactgtattttgtggattctgacccattgcaggatcacaatatgtataatgattcccaaggtggagatcttttccagttgttgatgcct

SEQ ID NO: 3 - DNA, 54 bp, Artificial Sequence
  ApoE tandem repeat (ApoEII)
ctgagaaagctgcggaagcggctgctgctgaggaagctgagaaaaagactgctg

SEQ ID NO: 4 - DNA, 63 bp, Artificial Sequence
  Linker
ctgggagggggaggatctggcggaggcggaagtggcggcggaggatcagggggcggaggctct

SEQ ID NO: 5 - protein, 550 aa, Artificial Sequence
  coIDS
MPPPRTGRGLLWLGLVLSSVCVALGSETQANSTTDALNVLLIIVDDLRPSLGCYGDKLVRSPNIDQLASHSLLFQNAFAQQAVCAPSRVSFLTGRRPDTTRLYDFNSYWRVHAGNFSTIPQYFKENGYVTMSVGKVFHPGISSNHTDDSPYSWSFPPYHPSSEKYENTKTCRGPDGELHANLLCPVDVLDVPEGTLPDKQSTEQAIQLLEKMKTSASPFFLAVGYHKPHIPFRYPKEFQKLYPLENITLAPDPEVPDGLPPVAYNPWMDIRQREDVQALNISVPYGPIPVDFQRKIRQSYFASVSYLDTQVGRLLSALDDLQLANSTIIAFTSDHGWALGEHGEWAKYSNFDVATHVPLIFYVPGRTASLPEAGEKLFPYLDPFDSASQLMEPGRQSMDLVELVSLFPTLAGLAGLQVPPRCPVPSFHVELCREGKNLLKHFRFRDLEEDPYLPGNPRELIAYSQYPRPSDIPQWNSDKPSLKDIKIMGYSIRTIDYRYTVWVGFNPDEFLANFSDIHAGELYFVDSDPLQDHNMYNDSQGGDLFQLLMP

SEQ ID NO: 6 - protein, 550 aa, Homo sapiens; identical to SEQ ID NO: 5

SEQ ID NO: 7 - protein, 18 aa, Artificial Sequence
  ApoE tandem repeat (ApoEII)
LRKLRKRLLLRKLRKRLL

SEQ ID NO: 8 - protein, 21 aa, Artificial Sequence
  Linker
LGGGGSGGGGSGGGGSGGGGS